European Patent Application EP 4 116 422 A1, published January 11, 2023. Title: DNA APTAMER SPECIFICALLY BINDING TO GLUTATHIONE AND USE OF THE SAME. Applicant: Nexmos Co., Ltd. The sequence listing filed with the application follows.

SEQUENCE LISTING (26 sequences)

SEQ ID NO: 1 - DNA, 30 bp, Artificial Sequence
  aptamer
gaccaacggaagcgcggcaccacaacggtg

SEQ ID NO: 2 - DNA, 43 bp, Artificial Sequence
  aptamer
cgaacagcatggaggcgcgcccgttgtgccgtgcgcgcgggat

SEQ ID NO: 3 - DNA, 43 bp, Artificial Sequence
  aptamer
ggcacgcagtgtgacgcgcctcgtcgttcactcggcgcgggat

SEQ ID NO: 4 - DNA, 43 bp, Artificial Sequence
  aptamer
gcacggcacaacgggcgcgcctccatgctgttcggcgcgggat

SEQ ID NO: 5 - DNA, 43 bp, Artificial Sequence
  aptamer
cgagtgaacgacgaggcgcgtcacactgcgtgccgcgcgggat

SEQ ID NO: 6 - DNA, 41 bp, Artificial Sequence
  aptamer
cgagtcagtgcgaggcgctcccctgtcggtgcgcgcgggat

SEQ ID NO: 7 - DNA, 41 bp, Artificial Sequence
  aptamer
gcaccgacaggggagcgcctcgcactgactcggcgcgggat

SEQ ID NO: 8 - DNA, 38 bp, Artificial Sequence
  aptamer
acgcatgccgggcgcgctccctgtcgtccgcgcgggat

SEQ ID NO: 9 - DNA, 29 bp, Artificial Sequence
  aptamer
cgactacgaggaggcgcgcaccacacgtt

SEQ ID NO: 10 - DNA, 38 bp, Artificial Sequence
  aptamer
aacgtacgtggagcggctccctgcactgcgcgcgggat

SEQ ID NO: 11 - DNA, 38 bp, Artificial Sequence
  aptamer
gcagtgcagggagccgctccacgtacgttgcgcgggat

SEQ ID NO: 12 - DNA, 39 bp, Artificial Sequence
  aptamer
ggtctgccggggccgcacctcctgtcgtcggcgcgggat

SEQ ID NO: 13 - DNA, 40 bp, Artificial Sequence
  aptamer
gcacaatcggggcgcgctcgtcctctggccggcgcgggat

SEQ ID NO: 14 - DNA, 40 bp, Artificial Sequence
  aptamer
cggccagaggacgagcgcgccccgattgtgcgcgcgggat

SEQ ID NO: 15 - DNA, 20 bp, Artificial Sequence
  aptamer
ggacgacagggagcgcgccc

SEQ ID NO: 16 - DNA, 39 bp, Artificial Sequence
  aptamer
cgacgacaggaggtgcggccccggcagaccgcgcgggat

SEQ ID NO: 17 - DNA, 43 bp, Artificial Sequence
  aptamer
cgagtgagggcgaggcgcgacgtcccttcggtccgcgcgggat

SEQ ID NO: 18 - DNA, 41 bp, Artificial Sequence
  aptamer
cgagtcagtgcgaggcgcgctcctgccgttgcgcgcgggat

SEQ ID NO: 19 - DNA, 43 bp, Artificial Sequence
  aptamer
ggaccgaagggacgtcgcgcctcgccctcactcggcgcgggat

SEQ ID NO: 20 - DNA, 28 bp, Artificial Sequence
  aptamer
cgacggagggaggcgcgcaccacacgtt

SEQ ID NO: 21 - DNA, 27 bp, Artificial Sequence
  aptamer
gaccaacggagcgcggcccacaacggt

SEQ ID NO: 22 - DNA, 25 bp, Artificial Sequence
  aptamer
gacatcaggagcgcgccccgtcacg

SEQ ID NO: 23 - DNA, 28 bp, Artificial Sequence
  aptamer
gaccaacggagcgcggcccacaacggtg

SEQ ID NO: 24 - DNA, 34 bp, Artificial Sequence
  Aptamer
cgaacagcatggaggcgcgcccgttgtgccgtgc

SEQ ID NO: 25 - DNA, 30 bp, Artificial Sequence
  Aptamer
cgagtgaacgacgaggcgcgtcacactgcg

SEQ ID NO: 26 - DNA, 30 bp, Artificial Sequence
  Aptamer
ggacgacagggagcgcgcccggcatgcgtg